European Patent Application EP 4 166 668 A1, published April 19, 2023. Title: NUCLEIC ACID MOLECULE TARGETING MITF GENE AND USE THEREOF. Applicant: Ractigen Therapeutics. The sequence listing filed with the application follows.

SEQUENCE LISTING (305 sequences)

SEQ ID NO: 1 - DNA, 500 bp, Homo sapiens
gcgaaggaaagttcttcctcgttgttccaatccgaggacaagctgatatgtcgcagcagcccagggaagcatgcgagctgataggaagtccttttattttaagacaggctcgaatgctaaaactttcttgtgccaaaacccttgactattttatttttaaaataagcacttggcgtgccctcgcagatgtctgagctgagaggtcggggcgatggtagaagagcagtcagtgtccattcttattcatattaagtagccaagtctgtacccttgaagcaagtggggagagaggagggagaggagctgctgacattgacaatgaatccaaacaggagttgcactagcggtgtccaccacgttgcctctcccccgcctggccttctgggagctgtagttttcgtgggagcggctccccaggcgagctgggaatgccccgcccgggccgaactacagatcccaggcggcgctcggccgccagcccctcccgcccgggtgcgagt

SEQ ID NO: 2 - DNA, 21 bp, Artificial Sequence
  MITF F1 Primer
cgacagaagaaactggagcac

SEQ ID NO: 3 - DNA, 22 bp, Artificial Sequence
  MITF R1 Primer
cccgtggatggaataagggaaa

SEQ ID NO: 4 - DNA, 21 bp, Artificial Sequence
  HPRT1 F Primer
aaagatggtcaaggtcgcaag

SEQ ID NO: 5 - DNA, 23 bp, Artificial Sequence
  HPRT1 R Primer
tagtcaagggcatatcctacaac

SEQ ID NO: 6 - DNA, 22 bp, Artificial Sequence
  TBP F Primer
tgctcacccaccaacaatttag

SEQ ID NO: 7 - DNA, 22 bp, Artificial Sequence
  TBP R Primer
tctgctctgactttagcacctg

SEQ ID NO: 8 - DNA, 19 bp, Artificial Sequence
  RAG4-500 Active Target Sequence
gcgaaggaaagttcttcct

SEQ ID NO: 9 - DNA, 19 bp, Artificial Sequence
  RAG4-498 Active Target Sequence
gaaggaaagttcttcctcg

SEQ ID NO: 10 - DNA, 19 bp, Artificial Sequence
  RAG4-497 Active Target Sequence
aaggaaagttcttcctcgt

SEQ ID NO: 11 - DNA, 19 bp, Artificial Sequence
  RAG4-494 Active Target Sequence
gaaagttcttcctcgttgt

SEQ ID NO: 12 - DNA, 19 bp, Artificial Sequence
  RAG4-491 Active Target Sequence
agttcttcctcgttgttcc

SEQ ID NO: 13 - DNA, 19 bp, Artificial Sequence
  RAG4-490 Active Target Sequence
gttcttcctcgttgttcca

SEQ ID NO: 14 - DNA, 19 bp, Artificial Sequence
  RAG4-489 Active Target Sequence
ttcttcctcgttgttccaa

SEQ ID NO: 15 - DNA, 19 bp, Artificial Sequence
  RAG4-487 Active Target Sequence
cttcctcgttgttccaatc

SEQ ID NO: 16 - DNA, 19 bp, Artificial Sequence
  RAG4-485 Active Target Sequence
tcctcgttgttccaatccg

SEQ ID NO: 17 - DNA, 19 bp, Artificial Sequence
  RAG4-483 Active Target Sequence
ctcgttgttccaatccgag

SEQ ID NO: 18 - DNA, 19 bp, Artificial Sequence
  RAG4-482 Active Target Sequence
tcgttgttccaatccgagg

SEQ ID NO: 19 - DNA, 19 bp, Artificial Sequence
  RAG4-481 Active Target Sequence
cgttgttccaatccgagga

SEQ ID NO: 20 - DNA, 19 bp, Artificial Sequence
  RAG4-479 Active Target Sequence
ttgttccaatccgaggaca

SEQ ID NO: 21 - DNA, 19 bp, Artificial Sequence
  RAG4-478 Active Target Sequence
tgttccaatccgaggacaa

SEQ ID NO: 22 - DNA, 19 bp, Artificial Sequence
  RAG4-477 Active Target Sequence
gttccaatccgaggacaag

SEQ ID NO: 23 - DNA, 19 bp, Artificial Sequence
  RAG4-476 Active Target Sequence
ttccaatccgaggacaagc

SEQ ID NO: 24 - DNA, 19 bp, Artificial Sequence
  RAG4-475 Active Target Sequence
tccaatccgaggacaagct

SEQ ID NO: 25 - DNA, 19 bp, Artificial Sequence
  RAG4-474 Active Target Sequence
ccaatccgaggacaagctg

SEQ ID NO: 26 - DNA, 19 bp, Artificial Sequence
  RAG4-473 Active Target Sequence
caatccgaggacaagctga

SEQ ID NO: 27 - DNA, 19 bp, Artificial Sequence
  RAG4-472 Active Target Sequence
aatccgaggacaagctgat

SEQ ID NO: 28 - DNA, 19 bp, Artificial Sequence
  RAG4-469 Active Target Sequence
ccgaggacaagctgatatg

SEQ ID NO: 29 - DNA, 19 bp, Artificial Sequence
  RAG4-467 Active Target Sequence
gaggacaagctgatatgtc

SEQ ID NO: 30 - DNA, 19 bp, Artificial Sequence
  RAG4-466 Active Target Sequence
aggacaagctgatatgtcg

SEQ ID NO: 31 - DNA, 19 bp, Artificial Sequence
  RAG4-464 Active Target Sequence
gacaagctgatatgtcgca

SEQ ID NO: 32 - DNA, 19 bp, Artificial Sequence
  RAG4-461 Active Target Sequence
aagctgatatgtcgcagca

SEQ ID NO: 33 - DNA, 19 bp, Artificial Sequence
  RAG4-460 Active Target Sequence
agctgatatgtcgcagcag

SEQ ID NO: 34 - DNA, 19 bp, Artificial Sequence
  RAG4-459 Active Target Sequence
gctgatatgtcgcagcagc

SEQ ID NO: 35 - DNA, 19 bp, Artificial Sequence
  RAG4-458 Active Target Sequence
ctgatatgtcgcagcagcc

SEQ ID NO: 36 - DNA, 19 bp, Artificial Sequence
  RAG4-456 Active Target Sequence
gatatgtcgcagcagccca

SEQ ID NO: 37 - DNA, 19 bp, Artificial Sequence
  RAG4-446 Active Target Sequence
agcagcccagggaagcatg

SEQ ID NO: 38 - DNA, 19 bp, Artificial Sequence
  RAG4-432 Active Target Sequence
gcatgcgagctgataggaa

SEQ ID NO: 39 - DNA, 19 bp, Artificial Sequence
  RAG4-431 Active Target Sequence
catgcgagctgataggaag

SEQ ID NO: 40 - DNA, 19 bp, Artificial Sequence
  RAG4-427 Active Target Sequence
cgagctgataggaagtcct

SEQ ID NO: 41 - DNA, 19 bp, Artificial Sequence
  RAG4-426 Active Target Sequence
gagctgataggaagtcctt

SEQ ID NO: 42 - DNA, 19 bp, Artificial Sequence
  RAG4-403 Active Target Sequence
tttaagacaggctcgaatg

SEQ ID NO: 43 - DNA, 19 bp, Artificial Sequence
  RAG4-402 Active Target Sequence
ttaagacaggctcgaatgc

SEQ ID NO: 44 - DNA, 19 bp, Artificial Sequence
  RAG4-401 Active Target Sequence
taagacaggctcgaatgct

SEQ ID NO: 45 - DNA, 19 bp, Artificial Sequence
  RAG4-396 Active Target Sequence
caggctcgaatgctaaaac

SEQ ID NO: 46 - DNA, 19 bp, Artificial Sequence
  RAG4-395 Active Target Sequence
aggctcgaatgctaaaact

SEQ ID NO: 47 - DNA, 19 bp, Artificial Sequence
  RAG4-394 Active Target Sequence
ggctcgaatgctaaaactt

SEQ ID NO: 48 - DNA, 19 bp, Artificial Sequence
  RAG4-385 Active Target Sequence
gctaaaactttcttgtgcc

SEQ ID NO: 49 - DNA, 19 bp, Artificial Sequence
  RAG4-375 Active Target Sequence
tcttgtgccaaaacccttg

SEQ ID NO: 50 - DNA, 19 bp, Artificial Sequence
  RAG4-374 Active Target Sequence
cttgtgccaaaacccttga

SEQ ID NO: 51 - DNA, 19 bp, Artificial Sequence
  RAG4-372 Active Target Sequence
tgtgccaaaacccttgact

SEQ ID NO: 52 - DNA, 19 bp, Artificial Sequence
  RAG4-371 Active Target Sequence
gtgccaaaacccttgacta

SEQ ID NO: 53 - DNA, 19 bp, Artificial Sequence
  RAG4-369 Active Target Sequence
gccaaaacccttgactatt

SEQ ID NO: 54 - DNA, 19 bp, Artificial Sequence
  RAG4-342 Active Target Sequence
aaaataagcacttggcgtg

SEQ ID NO: 55 - DNA, 19 bp, Artificial Sequence
  RAG4-341 Active Target Sequence
aaataagcacttggcgtgc

SEQ ID NO: 56 - DNA, 19 bp, Artificial Sequence
  RAG4-323 Active Target Sequence
ccctcgcagatgtctgagc

SEQ ID NO: 57 - DNA, 19 bp, Artificial Sequence
  RAG4-322 Active Target Sequence
cctcgcagatgtctgagct

SEQ ID NO: 58 - DNA, 19 bp, Artificial Sequence
  RAG4-320 Active Target Sequence
tcgcagatgtctgagctga

SEQ ID NO: 59 - DNA, 19 bp, Artificial Sequence
  RAG4-318 Active Target Sequence
gcagatgtctgagctgaga

SEQ ID NO: 60 - DNA, 19 bp, Artificial Sequence
  RAG4-317 Active Target Sequence
cagatgtctgagctgagag

SEQ ID NO: 61 - DNA, 19 bp, Artificial Sequence
  RAG4-316 Active Target Sequence
agatgtctgagctgagagg

SEQ ID NO: 62 - DNA, 19 bp, Artificial Sequence
  RAG4-298 Active Target Sequence
gtcggggcgatggtagaag

SEQ ID NO: 63 - DNA, 19 bp, Artificial Sequence
  RAG4-297 Active Target Sequence
tcggggcgatggtagaaga

SEQ ID NO: 64 - DNA, 19 bp, Artificial Sequence
  RAG4-296 Active Target Sequence
cggggcgatggtagaagag

SEQ ID NO: 65 - DNA, 19 bp, Artificial Sequence
  RAG4-295 Active Target Sequence
ggggcgatggtagaagagc

SEQ ID NO: 66 - DNA, 19 bp, Artificial Sequence
  RAG4-293 Active Target Sequence
ggcgatggtagaagagcag

SEQ ID NO: 67 - DNA, 19 bp, Artificial Sequence
  RAG4-292 Active Target Sequence
gcgatggtagaagagcagt

SEQ ID NO: 68 - DNA, 19 bp, Artificial Sequence
  RAG4-290 Active Target Sequence
gatggtagaagagcagtca

SEQ ID NO: 69 - DNA, 19 bp, Artificial Sequence
  RAG4-289 Active Target Sequence
atggtagaagagcagtcag

SEQ ID NO: 70 - DNA, 19 bp, Artificial Sequence
  RAG4-288 Active Target Sequence
tggtagaagagcagtcagt

SEQ ID NO: 71 - DNA, 19 bp, Artificial Sequence
  RAG4-285 Active Target Sequence
tagaagagcagtcagtgtc

SEQ ID NO: 72 - DNA, 19 bp, Artificial Sequence
  RAG4-284 Active Target Sequence
agaagagcagtcagtgtcc

SEQ ID NO: 73 - DNA, 19 bp, Artificial Sequence
  RAG4-283 Active Target Sequence
gaagagcagtcagtgtcca

SEQ ID NO: 74 - DNA, 19 bp, Artificial Sequence
  RAG4-282 Active Target Sequence
aagagcagtcagtgtccat

SEQ ID NO: 75 - DNA, 19 bp, Artificial Sequence
  RAG4-281 Active Target Sequence
agagcagtcagtgtccatt

SEQ ID NO: 76 - DNA, 19 bp, Artificial Sequence
  RAG4-280 Active Target Sequence
gagcagtcagtgtccattc

SEQ ID NO: 77 - DNA, 19 bp, Artificial Sequence
  RAG4-181 Active Target Sequence
tgaatccaaacaggagttg

SEQ ID NO: 78 - DNA, 19 bp, Artificial Sequence
  RAG4-180 Active Target Sequence
gaatccaaacaggagttgc

SEQ ID NO: 79 - DNA, 19 bp, Artificial Sequence
  RAG4-179 Active Target Sequence
aatccaaacaggagttgca

SEQ ID NO: 80 - DNA, 19 bp, Artificial Sequence
  RAG4-176 Active Target Sequence
ccaaacaggagttgcacta

SEQ ID NO: 81 - DNA, 19 bp, Artificial Sequence
  RAG4-175 Active Target Sequence
caaacaggagttgcactag

SEQ ID NO: 82 - DNA, 19 bp, Artificial Sequence
  RAG4-174 Active Target Sequence
aaacaggagttgcactagc

SEQ ID NO: 83 - DNA, 19 bp, Artificial Sequence
  RAG4-172 Active Target Sequence
acaggagttgcactagcgg

SEQ ID NO: 84 - DNA, 19 bp, Artificial Sequence
  RAG4-170 Active Target Sequence
aggagttgcactagcggtg

SEQ ID NO: 85 - DNA, 19 bp, Artificial Sequence
  RAG4-166 Active Target Sequence
gttgcactagcggtgtcca

SEQ ID NO: 86 - DNA, 19 bp, Artificial Sequence
  RAG4-165 Active Target Sequence
ttgcactagcggtgtccac

SEQ ID NO: 87 - DNA, 19 bp, Artificial Sequence
  RAG4-158 Active Target Sequence
agcggtgtccaccacgttg

SEQ ID NO: 88 - DNA, 19 bp, Artificial Sequence
  RAG4-249 Active Target Sequence
agtagccaagtctgtaccc

SEQ ID NO: 89 - DNA, 19 bp, Artificial Sequence
  RAG4-238 Active Target Sequence
ctgtacccttgaagcaagt

SEQ ID NO: 90 - DNA, 19 bp, Artificial Sequence
  RAG4-236 Active Target Sequence
gtacccttgaagcaagtgg

SEQ ID NO: 91 - DNA, 19 bp, Artificial Sequence
  RAG4-213 Active Target Sequence
agaggagggagaggagctg

SEQ ID NO: 92 - DNA, 19 bp, Artificial Sequence
  RAG4-211 Active Target Sequence
aggagggagaggagctgct

SEQ ID NO: 93 - DNA, 19 bp, Artificial Sequence
  RAG4-123 Active Target Sequence
ccttctgggagctgtagtt

SEQ ID NO: 94 - DNA, 19 bp, Artificial Sequence
  RAG4-116 Active Target Sequence
ggagctgtagttttcgtgg

SEQ ID NO: 95 - DNA, 19 bp, Artificial Sequence
  RAG4-115 Active Target Sequence
gagctgtagttttcgtggg

SEQ ID NO: 96 - DNA, 19 bp, Artificial Sequence
  RAG4-114 Active Target Sequence
agctgtagttttcgtggga

SEQ ID NO: 97 - DNA, 19 bp, Artificial Sequence
  RAG4-113 Active Target Sequence
gctgtagttttcgtgggag

SEQ ID NO: 98 - DNA, 19 bp, Artificial Sequence
  RAG4-111 Active Target Sequence
tgtagttttcgtgggagcg

SEQ ID NO: 99 - DNA, 19 bp, Artificial Sequence
  RAG4-109 Active Target Sequence
tagttttcgtgggagcggc

SEQ ID NO: 100 - DNA, 19 bp, Artificial Sequence
  RAG4-107 Active Target Sequence
gttttcgtgggagcggctc

SEQ ID NO: 101 - DNA, 19 bp, Artificial Sequence
  RAG4-62 Active Target Sequence
cgggccgaactacagatcc

SEQ ID NO: 102 - DNA, 19 bp, Artificial Sequence
  RAG4-61 Active Target Sequence
gggccgaactacagatccc

SEQ ID NO: 103 - DNA, 19 bp, Artificial Sequence
  RAG4-55 Active Target Sequence
aactacagatcccaggcgg

SEQ ID NO: 104 - DNA, 19 bp, Artificial Sequence
  RAG4-54 Active Target Sequence
actacagatcccaggcggc

SEQ ID NO: 105 - DNA, 21 bp, Artificial Sequence
  Synthetic DNA/RNA Functional saRNA sequence
gcgaaggaaaguucuuccutt

SEQ ID NO: 106 - DNA, 21 bp, Artificial Sequence
  Synthetic DNA/RNA Functional saRNA Sequence
gaaggaaaguucuuccucgtt

SEQ ID NO: 107 - DNA, 21 bp, Artificial Sequence
  Synthetic DNA/RNA Functional saRNA Sequence
aaggaaaguucuuccucgutt

SEQ ID NO: 108 - DNA, 21 bp, Artificial Sequence
  Synthetic DNA/RNA Functional saRNA Sequence
gaaaguucuuccucguugutt

SEQ ID NO: 109 - DNA, 21 bp, Artificial Sequence
  Synthetic DNA/RNA Functional saRNA Sequence
aguucuuccucguuguucctt

SEQ ID NO: 110 - DNA, 21 bp, Artificial Sequence
  Synthetic DNA/RNA Functional saRNA Sequence
guucuuccucguuguuccatt

SEQ ID NO: 111 - DNA, 21 bp, Artificial Sequence
  Synthetic DNA/RNA Functional saRNA Sequence
uucuuccucguuguuccaatt

SEQ ID NO: 112 - DNA, 21 bp, Artificial Sequence
  Synthetic DNA/RNA Functional saRNA Sequence
cuuccucguuguuccaauctt

SEQ ID NO: 113 - DNA, 21 bp, Artificial Sequence
  Synthetic DNA/RNA Functional saRNA Sequence
uccucguuguuccaauccgtt

SEQ ID NO: 114 - DNA, 21 bp, Artificial Sequence
  Synthetic DNA/RNA Functional saRNA Sequence
cucguuguuccaauccgagtt

SEQ ID NO: 115 - DNA, 21 bp, Artificial Sequence
  Synthetic DNA/RNA Functional saRNA Sequence
ucguuguuccaauccgaggtt

SEQ ID NO: 116 - DNA, 21 bp, Artificial Sequence
  Synthetic DNA/RNA Functional saRNA Sequence
cguuguuccaauccgaggatt

SEQ ID NO: 117 - DNA, 21 bp, Artificial Sequence
  Synthetic DNA/RNA Functional saRNA Sequence
uuguuccaauccgaggacatt

SEQ ID NO: 118 - DNA, 21 bp, Artificial Sequence
  Synthetic DNA/RNA Functional saRNA Sequence
uguuccaauccgaggacaatt

SEQ ID NO: 119 - DNA, 21 bp, Artificial Sequence
  Synthetic DNA/RNA Functional saRNA Sequence
guuccaauccgaggacaagtt

SEQ ID NO: 120 - DNA, 21 bp, Artificial Sequence
  Synthetic DNA/RNA Functional saRNA Sequence
uuccaauccgaggacaagctt

SEQ ID NO: 121 - DNA, 21 bp, Artificial Sequence
  Synthetic DNA/RNA Functional saRNA Sequence
uccaauccgaggacaagcutt

SEQ ID NO: 122 - DNA, 21 bp, Artificial Sequence
  Synthetic DNA/RNA Functional saRNA Sequence
ccaauccgaggacaagcugtt

SEQ ID NO: 123 - DNA, 21 bp, Artificial Sequence
  Synthetic DNA/RNA Functional saRNA Sequence
caauccgaggacaagcugatt

SEQ ID NO: 124 - DNA, 21 bp, Artificial Sequence
  Synthetic DNA/RNA Functional saRNA Sequence
aauccgaggacaagcugautt

SEQ ID NO: 125 - DNA, 21 bp, Artificial Sequence
  Synthetic DNA/RNA Functional saRNA Sequence
ccgaggacaagcugauaugtt

SEQ ID NO: 126 - DNA, 21 bp, Artificial Sequence
  Synthetic DNA/RNA Functional saRNA Sequence
gaggacaagcugauauguctt

SEQ ID NO: 127 - DNA, 21 bp, Artificial Sequence
  Synthetic DNA/RNA Functional saRNA Sequence
aggacaagcugauaugucgtt

SEQ ID NO: 128 - DNA, 21 bp, Artificial Sequence
  Synthetic DNA/RNA Functional saRNA Sequence
gacaagcugauaugucgcatt

SEQ ID NO: 129 - DNA, 21 bp, Artificial Sequence
  Synthetic DNA/RNA Functional saRNA Sequence
aagcugauaugucgcagcatt

SEQ ID NO: 130 - DNA, 21 bp, Artificial Sequence
  Synthetic DNA/RNA Functional saRNA Sequence
agcugauaugucgcagcagtt

SEQ ID NO: 131 - DNA, 21 bp, Artificial Sequence
  Synthetic DNA/RNA Functional saRNA Sequence
gcugauaugucgcagcagctt

SEQ ID NO: 132 - DNA, 21 bp, Artificial Sequence
  Synthetic DNA/RNA Functional saRNA Sequence
cugauaugucgcagcagcctt

SEQ ID NO: 133 - DNA, 21 bp, Artificial Sequence
  Synthetic DNA/RNA Functional saRNA Sequence
gauaugucgcagcagcccatt

SEQ ID NO: 134 - DNA, 21 bp, Artificial Sequence
  Synthetic DNA/RNA Functional saRNA Sequence
agcagcccagggaagcaugtt

SEQ ID NO: 135 - DNA, 21 bp, Artificial Sequence
  Synthetic DNA/RNA Functional saRNA Sequence
gcaugcgagcugauaggaatt

SEQ ID NO: 136 - DNA, 21 bp, Artificial Sequence
  Synthetic DNA/RNA Functional saRNA Sequence
caugcgagcugauaggaagtt

SEQ ID NO: 137 - DNA, 21 bp, Artificial Sequence
  Synthetic DNA/RNA Functional saRNA Sequence
cgagcugauaggaaguccutt

SEQ ID NO: 138 - DNA, 21 bp, Artificial Sequence
  Synthetic DNA/RNA Functional saRNA Sequence
gagcugauaggaaguccuutt

SEQ ID NO: 139 - DNA, 21 bp, Artificial Sequence
  Synthetic DNA/RNA Functional saRNA Sequence
uuuaagacaggcucgaaugtt

SEQ ID NO: 140 - DNA, 21 bp, Artificial Sequence
  Synthetic DNA/RNA Functional saRNA Sequence
uuaagacaggcucgaaugctt

SEQ ID NO: 141 - DNA, 21 bp, Artificial Sequence
  Synthetic DNA/RNA Functional saRNA Sequence
uaagacaggcucgaaugcutt

SEQ ID NO: 142 - DNA, 21 bp, Artificial Sequence
  Synthetic DNA/RNA Functional saRNA Sequence
caggcucgaaugcuaaaactt

SEQ ID NO: 143 - DNA, 21 bp, Artificial Sequence
  Synthetic DNA/RNA Functional saRNA Sequence
aggcucgaaugcuaaaacutt

SEQ ID NO: 144 - DNA, 21 bp, Artificial Sequence
  Synthetic DNA/RNA Functional saRNA Sequence
ggcucgaaugcuaaaacuutt

SEQ ID NO: 145 - DNA, 21 bp, Artificial Sequence
  Synthetic DNA/RNA Functional saRNA Sequence
gcuaaaacuuucuugugcctt

SEQ ID NO: 146 - DNA, 21 bp, Artificial Sequence
  Synthetic DNA/RNA Functional saRNA Sequence
ucuugugccaaaacccuugtt

SEQ ID NO: 147 - DNA, 21 bp, Artificial Sequence
  Synthetic DNA/RNA Functional saRNA Sequence
cuugugccaaaacccuugatt

SEQ ID NO: 148 - DNA, 21 bp, Artificial Sequence
  Synthetic DNA/RNA Functional saRNA Sequence
ugugccaaaacccuugacutt

SEQ ID NO: 149 - DNA, 21 bp, Artificial Sequence
  Synthetic DNA/RNA Functional saRNA Sequence
gugccaaaacccuugacuatt

SEQ ID NO: 150 - DNA, 21 bp, Artificial Sequence
  Synthetic DNA/RNA Functional saRNA Sequence
gccaaaacccuugacuauutt

SEQ ID NO: 151 - DNA, 21 bp, Artificial Sequence
  Synthetic DNA/RNA Functional saRNA Sequence
aaaauaagcacuuggcgugtt

SEQ ID NO: 152 - DNA, 21 bp, Artificial Sequence
  Synthetic DNA/RNA Functional saRNA Sequence
aaauaagcacuuggcgugctt

SEQ ID NO: 153 - DNA, 21 bp, Artificial Sequence
  Synthetic DNA/RNA Functional saRNA Sequence
cccucgcagaugucugagctt

SEQ ID NO: 154 - DNA, 21 bp, Artificial Sequence
  Synthetic DNA/RNA Functional saRNA Sequence
ccucgcagaugucugagcutt

SEQ ID NO: 155 - DNA, 21 bp, Artificial Sequence
  Synthetic DNA/RNA Functional saRNA Sequence
ucgcagaugucugagcugatt

SEQ ID NO: 156 - DNA, 21 bp, Artificial Sequence
  Synthetic DNA/RNA Functional saRNA Sequence
gcagaugucugagcugagatt

SEQ ID NO: 157 - DNA, 21 bp, Artificial Sequence
  Synthetic DNA/RNA Functional saRNA Sequence
cagaugucugagcugagagtt

SEQ ID NO: 158 - DNA, 21 bp, Artificial Sequence
  Synthetic DNA/RNA Functional saRNA Sequence
agaugucugagcugagaggtt

SEQ ID NO: 159 - DNA, 21 bp, Artificial Sequence
  Synthetic DNA/RNA Functional saRNA Sequence
gucggggcgaugguagaagtt

SEQ ID NO: 160 - DNA, 21 bp, Artificial Sequence
  Synthetic DNA/RNA Functional saRNA Sequence
ucggggcgaugguagaagatt

SEQ ID NO: 161 - DNA, 21 bp, Artificial Sequence
  Synthetic DNA/RNA Functional saRNA Sequence
cggggcgaugguagaagagtt

SEQ ID NO: 162 - DNA, 21 bp, Artificial Sequence
  Synthetic DNA/RNA Functional saRNA Sequence
ggggcgaugguagaagagctt

SEQ ID NO: 163 - DNA, 21 bp, Artificial Sequence
  Synthetic DNA/RNA Functional saRNA Sequence
ggcgaugguagaagagcagtt

SEQ ID NO: 164 - DNA, 21 bp, Artificial Sequence
  Synthetic DNA/RNA Functional saRNA Sequence
gcgaugguagaagagcagutt

SEQ ID NO: 165 - DNA, 21 bp, Artificial Sequence
  Synthetic DNA/RNA Functional saRNA Sequence
gaugguagaagagcagucatt

SEQ ID NO: 166 - DNA, 21 bp, Artificial Sequence
  Synthetic DNA/RNA Functional saRNA Sequence
augguagaagagcagucagtt

SEQ ID NO: 167 - DNA, 21 bp, Artificial Sequence
  Synthetic DNA/RNA Functional saRNA Sequence
ugguagaagagcagucagutt

SEQ ID NO: 168 - DNA, 21 bp, Artificial Sequence
  Synthetic DNA/RNA Functional saRNA Sequence
uagaagagcagucaguguctt

SEQ ID NO: 169 - DNA, 21 bp, Artificial Sequence
  Synthetic DNA/RNA Functional saRNA Sequence
agaagagcagucagugucctt

SEQ ID NO: 170 - DNA, 21 bp, Artificial Sequence
  Synthetic DNA/RNA Functional saRNA Sequence
gaagagcagucaguguccatt

SEQ ID NO: 171 - DNA, 21 bp, Artificial Sequence
  Synthetic DNA/RNA Functional saRNA Sequence
aagagcagucaguguccautt

SEQ ID NO: 172 - DNA, 21 bp, Artificial Sequence
  Synthetic DNA/RNA Functional saRNA Sequence
agagcagucaguguccauutt

SEQ ID NO: 173 - DNA, 21 bp, Artificial Sequence
  Synthetic DNA/RNA Functional saRNA Sequence
gagcagucaguguccauuctt

SEQ ID NO: 174 - DNA, 21 bp, Artificial Sequence
  Synthetic DNA/RNA Functional saRNA Sequence
ugaauccaaacaggaguugtt

SEQ ID NO: 175 - DNA, 21 bp, Artificial Sequence
  Synthetic DNA/RNA Functional saRNA Sequence
gaauccaaacaggaguugctt

SEQ ID NO: 176 - DNA, 21 bp, Artificial Sequence
  Synthetic DNA/RNA Functional saRNA Sequence
aauccaaacaggaguugcatt

SEQ ID NO: 177 - DNA, 21 bp, Artificial Sequence
  Synthetic DNA/RNA Functional saRNA Sequence
ccaaacaggaguugcacuatt

SEQ ID NO: 178 - DNA, 21 bp, Artificial Sequence
  Synthetic DNA/RNA Functional saRNA Sequence
caaacaggaguugcacuagtt

SEQ ID NO: 179 - DNA, 21 bp, Artificial Sequence
  Synthetic DNA/RNA Functional saRNA Sequence
aaacaggaguugcacuagctt

SEQ ID NO: 180 - DNA, 21 bp, Artificial Sequence
  Synthetic DNA/RNA Functional saRNA Sequence
acaggaguugcacuagcggtt

SEQ ID NO: 181 - DNA, 21 bp, Artificial Sequence
  Synthetic DNA/RNA Functional saRNA Sequence
aggaguugcacuagcggugtt

SEQ ID NO: 182 - DNA, 21 bp, Artificial Sequence
  Synthetic DNA/RNA Functional saRNA Sequence
guugcacuagcgguguccatt

SEQ ID NO: 183 - DNA, 21 bp, Artificial Sequence
  Synthetic DNA/RNA Functional saRNA Sequence
uugcacuagcgguguccactt

SEQ ID NO: 184 - DNA, 21 bp, Artificial Sequence
  Synthetic DNA/RNA Functional saRNA Sequence
agcgguguccaccacguugtt

SEQ ID NO: 185 - DNA, 21 bp, Artificial Sequence
  Synthetic DNA/RNA Functional saRNA Sequence
aguagccaagucuguaccctt

SEQ ID NO: 186 - DNA, 21 bp, Artificial Sequence
  Synthetic DNA/RNA Functional saRNA Sequence
cuguacccuugaagcaagutt

SEQ ID NO: 187 - DNA, 21 bp, Artificial Sequence
  Synthetic DNA/RNA Functional saRNA Sequence
guacccuugaagcaaguggtt

SEQ ID NO: 188 - DNA, 21 bp, Artificial Sequence
  Synthetic DNA/RNA Functional saRNA Sequence
agaggagggagaggagcugtt

SEQ ID NO: 189 - DNA, 21 bp, Artificial Sequence
  Synthetic DNA/RNA Functional saRNA Sequence
aggagggagaggagcugcutt

SEQ ID NO: 190 - DNA, 21 bp, Artificial Sequence
  Synthetic DNA/RNA Functional saRNA Sequence
ccuucugggagcuguaguutt

SEQ ID NO: 191 - DNA, 21 bp, Artificial Sequence
  Synthetic DNA/RNA Functional saRNA Sequence
ggagcuguaguuuucguggtt

SEQ ID NO: 192 - DNA, 21 bp, Artificial Sequence
  Synthetic DNA/RNA Functional saRNA Sequence
gagcuguaguuuucgugggtt

SEQ ID NO: 193 - DNA, 21 bp, Artificial Sequence
  Synthetic DNA/RNA Functional saRNA Sequence
agcuguaguuuucgugggatt

SEQ ID NO: 194 - DNA, 21 bp, Artificial Sequence
  Synthetic DNA/RNA Functional saRNA Sequence
gcuguaguuuucgugggagtt

SEQ ID NO: 195 - DNA, 21 bp, Artificial Sequence
  Synthetic DNA/RNA Functional saRNA Sequence
uguaguuuucgugggagcgtt

SEQ ID NO: 196 - DNA, 21 bp, Artificial Sequence
  Synthetic DNA/RNA Functional saRNA Sequence
uaguuuucgugggagcggctt

SEQ ID NO: 197 - DNA, 21 bp, Artificial Sequence
  Synthetic DNA/RNA Functional saRNA Sequence
guuuucgugggagcggcuctt

SEQ ID NO: 198 - DNA, 21 bp, Artificial Sequence
  Synthetic DNA/RNA Functional saRNA Sequence
cgggccgaacuacagaucctt

SEQ ID NO: 199 - DNA, 21 bp, Artificial Sequence
  Synthetic DNA/RNA Functional saRNA Sequence
gggccgaacuacagauccctt

SEQ ID NO: 200 - DNA, 21 bp, Artificial Sequence
  Synthetic DNA/RNA Functional saRNA Sequence
aacuacagaucccaggcggtt

SEQ ID NO: 201 - DNA, 21 bp, Artificial Sequence
  Synthetic DNA/RNA Functional saRNA Sequence
acuacagaucccaggcggctt

SEQ ID NO: 202 - DNA, 21 bp, Artificial Sequence
  Synthetic DNA/RNA Functional saRNA Sequence
aggaagaacuuuccuucgctt

SEQ ID NO: 203 - DNA, 21 bp, Artificial Sequence
  Synthetic DNA/RNA Functional saRNA Sequence
cgaggaagaacuuuccuuctt

SEQ ID NO: 204 - DNA, 21 bp, Artificial Sequence
  Synthetic DNA/RNA Functional saRNA Sequence
acgaggaagaacuuuccuutt

SEQ ID NO: 205 - DNA, 21 bp, Artificial Sequence
  Synthetic DNA/RNA Functional saRNA Sequence
acaacgaggaagaacuuuctt

SEQ ID NO: 206 - DNA, 21 bp, Artificial Sequence
  Synthetic DNA/RNA Functional saRNA Sequence
ggaacaacgaggaagaacutt

SEQ ID NO: 207 - DNA, 21 bp, Artificial Sequence
  Synthetic DNA/RNA Functional saRNA Sequence
uggaacaacgaggaagaactt

SEQ ID NO: 208 - DNA, 21 bp, Artificial Sequence
  Synthetic DNA/RNA Functional saRNA Sequence
uuggaacaacgaggaagaatt

SEQ ID NO: 209 - DNA, 21 bp, Artificial Sequence
  Synthetic DNA/RNA Functional saRNA Sequence
gauuggaacaacgaggaagtt

SEQ ID NO: 210 - DNA, 21 bp, Artificial Sequence
  Synthetic DNA/RNA Functional saRNA Sequence
cggauuggaacaacgaggatt

SEQ ID NO: 211 - DNA, 21 bp, Artificial Sequence
  Synthetic DNA/RNA Functional saRNA Sequence
cucggauuggaacaacgagtt

SEQ ID NO: 212 - DNA, 21 bp, Artificial Sequence
  Synthetic DNA/RNA Functional saRNA Sequence
ccucggauuggaacaacgatt

SEQ ID NO: 213 - DNA, 21 bp, Artificial Sequence
  Synthetic DNA/RNA Functional saRNA Sequence
uccucggauuggaacaacgtt

SEQ ID NO: 214 - DNA, 21 bp, Artificial Sequence
  Synthetic DNA/RNA Functional saRNA Sequence
uguccucggauuggaacaatt

SEQ ID NO: 215 - DNA, 21 bp, Artificial Sequence
  Synthetic DNA/RNA Functional saRNA Sequence
uuguccucggauuggaacatt

SEQ ID NO: 216 - DNA, 21 bp, Artificial Sequence
  Synthetic DNA/RNA Functional saRNA Sequence
cuuguccucggauuggaactt

SEQ ID NO: 217 - DNA, 21 bp, Artificial Sequence
  Synthetic DNA/RNA Functional saRNA Sequence
gcuuguccucggauuggaatt

SEQ ID NO: 218 - DNA, 21 bp, Artificial Sequence
  Synthetic DNA/RNA Functional saRNA Sequence
agcuuguccucggauuggatt

SEQ ID NO: 219 - DNA, 21 bp, Artificial Sequence
  Synthetic DNA/RNA Functional saRNA Sequence
cagcuuguccucggauuggtt

SEQ ID NO: 220 - DNA, 21 bp, Artificial Sequence
  Synthetic DNA/RNA Functional saRNA Sequence
ucagcuuguccucggauugtt

SEQ ID NO: 221 - DNA, 21 bp, Artificial Sequence
  Synthetic DNA/RNA Functional saRNA Sequence
aucagcuuguccucggauutt

SEQ ID NO: 222 - DNA, 21 bp, Artificial Sequence
  Synthetic DNA/RNA Functional saRNA Sequence
cauaucagcuuguccucggtt

SEQ ID NO: 223 - DNA, 21 bp, Artificial Sequence
  Synthetic DNA/RNA Functional saRNA Sequence
gacauaucagcuuguccuctt

SEQ ID NO: 224 - DNA, 21 bp, Artificial Sequence
  Synthetic DNA/RNA Functional saRNA Sequence
cgacauaucagcuuguccutt

SEQ ID NO: 225 - DNA, 21 bp, Artificial Sequence
  Synthetic DNA/RNA Functional saRNA Sequence
ugcgacauaucagcuuguctt

SEQ ID NO: 226 - DNA, 21 bp, Artificial Sequence
  Synthetic DNA/RNA Functional saRNA Sequence
ugcugcgacauaucagcuutt

SEQ ID NO: 227 - DNA, 21 bp, Artificial Sequence
  Synthetic DNA/RNA Functional saRNA Sequence
cugcugcgacauaucagcutt

SEQ ID NO: 228 - DNA, 21 bp, Artificial Sequence
  Synthetic DNA/RNA Functional saRNA Sequence
gcugcugcgacauaucagctt

SEQ ID NO: 229 - DNA, 21 bp, Artificial Sequence
  Synthetic DNA/RNA Functional saRNA Sequence
ggcugcugcgacauaucagtt

SEQ ID NO: 230 - DNA, 21 bp, Artificial Sequence
  Synthetic DNA/RNA Functional saRNA Sequence
ugggcugcugcgacauauctt

SEQ ID NO: 231 - DNA, 21 bp, Artificial Sequence
  Synthetic DNA/RNA Functional saRNA Sequence
caugcuucccugggcugcutt

SEQ ID NO: 232 - DNA, 21 bp, Artificial Sequence
  Synthetic DNA/RNA Functional saRNA Sequence
uuccuaucagcucgcaugctt

SEQ ID NO: 233 - DNA, 21 bp, Artificial Sequence
  Synthetic DNA/RNA Functional saRNA Sequence
cuuccuaucagcucgcaugtt

SEQ ID NO: 234 - DNA, 21 bp, Artificial Sequence
  Synthetic DNA/RNA Functional saRNA Sequence
aggacuuccuaucagcucgtt

SEQ ID NO: 235 - DNA, 21 bp, Artificial Sequence
  Synthetic DNA/RNA Functional saRNA Sequence
aaggacuuccuaucagcuctt

SEQ ID NO: 236 - DNA, 21 bp, Artificial Sequence
  Synthetic DNA/RNA Functional saRNA Sequence
cauucgagccugucuuaaatt

SEQ ID NO: 237 - DNA, 21 bp, Artificial Sequence
  Synthetic DNA/RNA Functional saRNA Sequence
gcauucgagccugucuuaatt

SEQ ID NO: 238 - DNA, 21 bp, Artificial Sequence
  Synthetic DNA/RNA Functional saRNA Sequence
agcauucgagccugucuuatt

SEQ ID NO: 239 - DNA, 21 bp, Artificial Sequence
  Synthetic DNA/RNA Functional saRNA Sequence
guuuuagcauucgagccugtt

SEQ ID NO: 240 - DNA, 21 bp, Artificial Sequence
  Synthetic DNA/RNA Functional saRNA Sequence
aguuuuagcauucgagccutt

SEQ ID NO: 241 - DNA, 21 bp, Artificial Sequence
  Synthetic DNA/RNA Functional saRNA Sequence
aaguuuuagcauucgagcctt

SEQ ID NO: 242 - DNA, 21 bp, Artificial Sequence
  Synthetic DNA/RNA Functional saRNA Sequence
ggcacaagaaaguuuuagctt

SEQ ID NO: 243 - DNA, 21 bp, Artificial Sequence
  Synthetic DNA/RNA Functional saRNA Sequence
caaggguuuuggcacaagatt

SEQ ID NO: 244 - DNA, 21 bp, Artificial Sequence
  Synthetic DNA/RNA Functional saRNA Sequence
ucaaggguuuuggcacaagtt

SEQ ID NO: 245 - DNA, 21 bp, Artificial Sequence
  Synthetic DNA/RNA Functional saRNA Sequence
agucaaggguuuuggcacatt

SEQ ID NO: 246 - DNA, 21 bp, Artificial Sequence
  Synthetic DNA/RNA Functional saRNA Sequence
uagucaaggguuuuggcactt

SEQ ID NO: 247 - DNA, 21 bp, Artificial Sequence
  Synthetic DNA/RNA Functional saRNA Sequence
aauagucaaggguuuuggctt

SEQ ID NO: 248 - DNA, 21 bp, Artificial Sequence
  Synthetic DNA/RNA Functional saRNA Sequence
cacgccaagugcuuauuuutt

SEQ ID NO: 249 - DNA, 21 bp, Artificial Sequence
  Synthetic DNA/RNA Functional saRNA Sequence
gcacgccaagugcuuauuutt

SEQ ID NO: 250 - DNA, 21 bp, Artificial Sequence
  Synthetic DNA/RNA Functional saRNA Sequence
gcucagacaucugcgagggtt

SEQ ID NO: 251 - DNA, 21 bp, Artificial Sequence
  Synthetic DNA/RNA Functional saRNA Sequence
agcucagacaucugcgaggtt

SEQ ID NO: 252 - DNA, 21 bp, Artificial Sequence
  Synthetic DNA/RNA Functional saRNA Sequence
ucagcucagacaucugcgatt

SEQ ID NO: 253 - DNA, 21 bp, Artificial Sequence
  Synthetic DNA/RNA Functional saRNA Sequence
ucucagcucagacaucugctt

SEQ ID NO: 254 - DNA, 21 bp, Artificial Sequence
  Synthetic DNA/RNA Functional saRNA Sequence
cucucagcucagacaucugtt

SEQ ID NO: 255 - DNA, 21 bp, Artificial Sequence
  Synthetic DNA/RNA Functional saRNA Sequence
ccucucagcucagacaucutt

SEQ ID NO: 256 - DNA, 21 bp, Artificial Sequence
  Synthetic DNA/RNA Functional saRNA Sequence
cuucuaccaucgccccgactt

SEQ ID NO: 257 - DNA, 21 bp, Artificial Sequence
  Synthetic DNA/RNA Functional saRNA Sequence
ucuucuaccaucgccccgatt

SEQ ID NO: 258 - DNA, 21 bp, Artificial Sequence
  Synthetic DNA/RNA Functional saRNA Sequence
cucuucuaccaucgccccgtt

SEQ ID NO: 259 - DNA, 21 bp, Artificial Sequence
  Synthetic DNA/RNA Functional saRNA Sequence
gcucuucuaccaucgcccctt

SEQ ID NO: 260 - DNA, 21 bp, Artificial Sequence
  Synthetic DNA/RNA Functional saRNA Sequence
cugcucuucuaccaucgcctt

SEQ ID NO: 261 - DNA, 21 bp, Artificial Sequence
  Synthetic DNA/RNA Functional saRNA Sequence
acugcucuucuaccaucgctt

SEQ ID NO: 262 - DNA, 21 bp, Artificial Sequence
  Synthetic DNA/RNA Functional saRNA Sequence
ugacugcucuucuaccauctt

SEQ ID NO: 263 - DNA, 21 bp, Artificial Sequence
  Synthetic DNA/RNA Functional saRNA Sequence
cugacugcucuucuaccautt

SEQ ID NO: 264 - DNA, 21 bp, Artificial Sequence
  Synthetic DNA/RNA Functional saRNA Sequence
acugacugcucuucuaccatt

SEQ ID NO: 265 - DNA, 21 bp, Artificial Sequence
  Synthetic DNA/RNA Functional saRNA Sequence
gacacugacugcucuucuatt

SEQ ID NO: 266 - DNA, 21 bp, Artificial Sequence
  Synthetic DNA/RNA Functional saRNA Sequence
ggacacugacugcucuucutt

SEQ ID NO: 267 - DNA, 21 bp, Artificial Sequence
  Synthetic DNA/RNA Functional saRNA Sequence
uggacacugacugcucuuctt

SEQ ID NO: 268 - DNA, 21 bp, Artificial Sequence
  Synthetic DNA/RNA Functional saRNA Sequence
auggacacugacugcucuutt

SEQ ID NO: 269 - DNA, 21 bp, Artificial Sequence
  Synthetic DNA/RNA Functional saRNA Sequence
aauggacacugacugcucutt

SEQ ID NO: 270 - DNA, 21 bp, Artificial Sequence
  Synthetic DNA/RNA Functional saRNA Sequence
gaauggacacugacugcuctt

SEQ ID NO: 271 - DNA, 21 bp, Artificial Sequence
  Synthetic DNA/RNA Functional saRNA Sequence
caacuccuguuuggauucatt

SEQ ID NO: 272 - DNA, 21 bp, Artificial Sequence
  Synthetic DNA/RNA Functional saRNA Sequence
gcaacuccuguuuggauuctt

SEQ ID NO: 273 - DNA, 21 bp, Artificial Sequence
  Synthetic DNA/RNA Functional saRNA Sequence
ugcaacuccuguuuggauutt

SEQ ID NO: 274 - DNA, 21 bp, Artificial Sequence
  Synthetic DNA/RNA Functional saRNA Sequence
uagugcaacuccuguuuggtt

SEQ ID NO: 275 - DNA, 21 bp, Artificial Sequence
  Synthetic DNA/RNA Functional saRNA Sequence
cuagugcaacuccuguuugtt

SEQ ID NO: 276 - DNA, 21 bp, Artificial Sequence
  Synthetic DNA/RNA Functional saRNA Sequence
gcuagugcaacuccuguuutt

SEQ ID NO: 277 - DNA, 21 bp, Artificial Sequence
  Synthetic DNA/RNA Functional saRNA Sequence
ccgcuagugcaacuccugutt

SEQ ID NO: 278 - DNA, 21 bp, Artificial Sequence
  Synthetic DNA/RNA Functional saRNA Sequence
caccgcuagugcaacuccutt

SEQ ID NO: 279 - DNA, 21 bp, Artificial Sequence
  Synthetic DNA/RNA Functional saRNA Sequence
uggacaccgcuagugcaactt

SEQ ID NO: 280 - DNA, 21 bp, Artificial Sequence
  Synthetic DNA/RNA Functional saRNA Sequence
guggacaccgcuagugcaatt

SEQ ID NO: 281 - DNA, 21 bp, Artificial Sequence
  Synthetic DNA/RNA Functional saRNA Sequence
caacgugguggacaccgcutt

SEQ ID NO: 282 - DNA, 21 bp, Artificial Sequence
  Synthetic DNA/RNA Functional saRNA Sequence
ggguacagacuuggcuacutt

SEQ ID NO: 283 - DNA, 21 bp, Artificial Sequence
  Synthetic DNA/RNA Functional saRNA Sequence
acuugcuucaaggguacagtt

SEQ ID NO: 284 - DNA, 21 bp, Artificial Sequence
  Synthetic DNA/RNA Functional saRNA Sequence
ccacuugcuucaaggguactt

SEQ ID NO: 285 - DNA, 21 bp, Artificial Sequence
  Synthetic DNA/RNA Functional saRNA Sequence
cagcuccucucccuccucutt

SEQ ID NO: 286 - DNA, 21 bp, Artificial Sequence
  Synthetic DNA/RNA Functional saRNA Sequence
agcagcuccucucccuccutt

SEQ ID NO: 287 - DNA, 21 bp, Artificial Sequence
  Synthetic DNA/RNA Functional saRNA Sequence
aacuacagcucccagaaggtt

SEQ ID NO: 288 - DNA, 21 bp, Artificial Sequence
  Synthetic DNA/RNA Functional saRNA Sequence
ccacgaaaacuacagcucctt

SEQ ID NO: 289 - DNA, 21 bp, Artificial Sequence
  Synthetic DNA/RNA Functional saRNA Sequence
cccacgaaaacuacagcuctt

SEQ ID NO: 290 - DNA, 21 bp, Artificial Sequence
  Synthetic DNA/RNA Functional saRNA Sequence
ucccacgaaaacuacagcutt

SEQ ID NO: 291 - DNA, 21 bp, Artificial Sequence
  Synthetic DNA/RNA Functional saRNA Sequence
cucccacgaaaacuacagctt

SEQ ID NO: 292 - DNA, 21 bp, Artificial Sequence
  Synthetic DNA/RNA Functional saRNA Sequence
cgcucccacgaaaacuacatt

SEQ ID NO: 293 - DNA, 21 bp, Artificial Sequence
  Synthetic DNA/RNA Functional saRNA Sequence
gccgcucccacgaaaacuatt

SEQ ID NO: 294 - DNA, 21 bp, Artificial Sequence
  Synthetic DNA/RNA Functional saRNA Sequence
gagccgcucccacgaaaactt

SEQ ID NO: 295 - DNA, 21 bp, Artificial Sequence
  Synthetic DNA/RNA Functional saRNA Sequence
ggaucuguaguucggcccgtt

SEQ ID NO: 296 - DNA, 21 bp, Artificial Sequence
  Synthetic DNA/RNA Functional saRNA Sequence
gggaucuguaguucggccctt

SEQ ID NO: 297 - DNA, 21 bp, Artificial Sequence
  Synthetic DNA/RNA Functional saRNA Sequence
ccgccugggaucuguaguutt

SEQ ID NO: 298 - DNA, 21 bp, Artificial Sequence
  Synthetic DNA/RNA Functional saRNA Sequence
gccgccugggaucuguagutt

SEQ ID NO: 299 - DNA, 93 bp, Artificial Sequence
  Hot spot region H1 (-500/-408)
gcgaaggaaagttcttcctcgttgttccaatccgaggacaagctgatatgtcgcagcagcccagggaagcatgcgagctgataggaagtcctt

SEQ ID NO: 300 - DNA, 53 bp, Artificial Sequence
  Hot spot region H2 (-403/-351)
tttaagacaggctcgaatgctaaaactttcttgtgccaaaacccttgactatt

SEQ ID NO: 301 - DNA, 81 bp, Artificial Sequence
  Hot spot region H3 (-342/-262)
aaaataagcacttggcgtgccctcgcagatgtctgagctgagaggtcggggcgatggtagaagagcagtcagtgtccattc

SEQ ID NO: 302 - DNA, 42 bp, Artificial Sequence
  Hot spot region H4 (-181/-140)
tgaatccaaacaggagttgcactagcggtgtccaccacgttg

SEQ ID NO: 303 - DNA, 57 bp, Artificial Sequence
  Warm spot region W1 (-249/-193)
agtagccaagtctgtacccttgaagcaagtggggagagaggagggagaggagctgct

SEQ ID NO: 304 - DNA, 35 bp, Artificial Sequence
  Warm spot region W2 (-123/-89)
ccttctgggagctgtagttttcgtgggagcggctc

SEQ ID NO: 305 - DNA, 27 bp, Artificial Sequence
  Warm spot region W3 (-62/-36)
cgggccgaactacagatcccaggcggc